European Patent Application EP 4 180 456 A1, published May 17, 2023. Title: Antibody binding to hepatitis B virus surface antigen and application of antibody. Applicant: Beijing Kawin Technology Share-holding Co., LTD. The sequence listing filed with the application follows.

SEQUENCE LISTING (48 sequences)

SEQ ID NO: 1 - protein, 123 aa, Artificial sequence
  VH of 021 and 079
QVQLVESGAEVKKPGASVKVSCKASGYTFTGYYMHWVRQAPGQGLEWMGWINPNSGGTNYAQKFQGRVTMTRDTSISTAYMELSRLRSDDTAVYYCARDLWNDDVDYYGMDVWGKGTLVTVSS

SEQ ID NO: 2 - protein, 123 aa, Artificial sequence
  VH of 005, 095, 096
EVQLVQSGAEVKKPGASVKVSCKASGYTFTGYYMHWVRQAPGQGLEWMGWINPNSGGTNYAQKFQGRVTMTRDTSISTAYMELSRLRSDDTAVYYCARDLWNDDVDYYGMDVWGQGTMVTVSS

SEQ ID NO: 3 - protein, 123 aa, Artificial sequence
  VH of 062
EVQLVESGAEVKKPGASVKVSCKASGYTFTGYYMHWVRQAPGQGLEWMGWINPNSGGTNYAQKFQGRVTMTRDTSISTAYMELSRLRSDDTAVYYCARDLWNDDVDYYGMDVWGQGTLVTVSS

SEQ ID NO: 4 - protein, 123 aa, Artificial sequence
  VH of 088
QITLKESGAEVKKPGASVKVSCKASGYSFIGYYLHWVRQAPGQGLEWMGWINPYNGGTNYAQKFQGRVTMTRDTSISTAYMELSRLRSDDTAVYYCARDLWNDDVDYYGMDVWGKGTLVTVSS

SEQ ID NO: 5 - protein, 123 aa, Artificial sequence
  VH of 090, 091, 093
EVQLVQSGAEVKKPGASMKVSCKASGYTFTDYYIHWVRQAPGQGPEWMGWINPNSGGTNYAQKFQGRVTMTRDTSISTAYMELSRLRSDDTAVYYCARDLWNDDVDYYGMDVWGKGTMVTVSS

SEQ ID NO: 6 - protein, 123 aa, Artificial sequence
  VH of 083
EVQLVQSGAEVKKPGASVKVSCKASGYTFTYYYMHWVRQAPGQGLEWMGWINPNSGGTNYAQKFQGRVTITADKSTSTAYMELSSLRSEDTAVYYCARDVWQQGGYYYYMDVWGKGTLVTVSS

SEQ ID NO: 7 - protein, 108 aa, Artificial sequence
  VL of 021, 083
DIQLTQSPSSLSASVGDRVTITCRASQSISTYLNWYQQKPGKAPKLLIYAASSLQSGVPSRFSGSGSGTDFTLTISSLQPEDFATYYCQQSYSTPLTFGGGTKVDIKR

SEQ ID NO: 8 - protein, 108 aa, Artificial sequence
  VL of 005, 062, 079, 088
DIQLTQSPSSLSASVGDRVTITCRASQSISSYLNWYQQKPGKAPKLLIYAASSLQSGVPSRFSGSGSGTDFTLTISSLQPEDFATYYCQQSYSTPLTFGGGTKLEIKR

SEQ ID NO: 9 - protein, 108 aa, Artificial sequence
  VL of 090
EIVLTQSPGTLSLSPGERATLSCRASQSVSSYLAWYQQKPGQAPRLLIYGASSRATGIPARFSGSGSGTEFTLTISSLQSEDFATYYCQQSYSTPLTFGPGTKVEIKR

SEQ ID NO: 10 - protein, 108 aa, Artificial sequence
  VL of 091
EIVLTQSPATLSLSPGERATLSCRASQSVSSYLAWYQQKPGQAPRLLIYDASNRATGIPARFSGSGSGTDFTLTISSLEPEDFATYYCQQSYSTPLTFGGGTKVDIKR

SEQ ID NO: 11 - protein, 108 aa, Artificial sequence
  VL of 093
DIQLTQSPSSLSASVGDRVTITCRASQSISSYLNWYQQKPGKAPKLLIYDASSLQSGVPSRFSGSGSGTEFTLTIRSLQPEDFATYYCQQSYSTPLTFGGGTKLEIKR

SEQ ID NO: 12 - protein, 108 aa, Artificial sequence
  VL of 095
DIQLTQSPSSLSASVGDRVTITCRASQSISSYLNWYQQKPGKAPKLLISAASSLQSGVPSRFSGSGSGTDFTLTISSLQPGDLATYYCQQSYSTPLTFGGGTKVEIKR

SEQ ID NO: 13 - protein, 108 aa, Artificial sequence
  VL of 096
ETTLTQSPSTLSASVGDRVTITCRASQSISSYLNWYQQKPGKAPQLLIYTASSLQSGVPSRFSGSGSGTDFTLTISSLQPEDFATYYCQQSYSTPLTFGQGTRLEIKR

SEQ ID NO: 14 - protein, 330 aa, Artificial sequence
  heavy chain constant region of humanized IgG1
ASTKGPSVFPLAPSSKSTSGGTAALGCLVKDYFPEPVTVSWNSGALTSGVHTFPAVLQSSGLYSLSSVVTVPSSSLGTQTYICNVNHKPSNTKVDKRVEPKSCDKTHTCPPCPAPELLGGPSVFLFPPKPKDTLMISRTPEVTCVVVDVSHEDPEVKFNWYVDGVEVHNAKTKPREEQYNSTYRVVSVLTVLHQDWLNGKEYKCKVSNKALPAPIEKTISKAKGQPREPQVYTLPPSREEMTKNQVSLTCLVKGFYPSDIAVEWESNGQPENNYKTTPPVLDSDGSFFLYSKLTVDKSRWQQGNVFSCSVMHEALHNHYTQKSLSLSPGK

SEQ ID NO: 15 - protein, 106 aa, Artificial sequence
  light chain constant region of humanized IgG1
TVAAPSVFIFPPSDEQLKSGTASVVCLLNNFYPREAKVQWKVDNALQSGNSQESVTEQDSKDSTYSLSSTLTLSKADYEKHKVYACEVTHQGLSSPVTKSFNRGEC

SEQ ID NO: 16 - protein, 232 aa, Artificial sequence
  sequence comprising HBsAg protein
MENTTSGFLGPLLVLQAGFFLLTRILTIPQSLDSWWTSLNFLGGAPTCPGQNSQSPTSNHSPTSCPPICPGYRWMCLRRFIIFLFILLLCLIFLLVLLDYQGMLPVCPLLPGTSTTSTGPCKTCTIPAQGTSMFPSCCCTKPSDGNCTCIPIPSSWAFARFLWEWASVRFSWLSLLVPFVQWFVGLSPTVWLSVIWMMWYWGPSLYNILSPFLPLLPIFFCLWVYIHHHHHH

SEQ ID NO: 17 - protein, 8 aa, Artificial sequence
  HCDR1
GYTFTGYY

SEQ ID NO: 18 - protein, 8 aa, Artificial sequence
  HCDR1
GYSFIGYY

SEQ ID NO: 19 - protein, 8 aa, Artificial sequence
  HCDR1
GYTFTDYY

SEQ ID NO: 20 - protein, 8 aa, Artificial sequence
  HCDR1
GYTFTYYY

SEQ ID NO: 21 - protein, 8 aa, Artificial sequence
  HCDR2
INPNSGGT

SEQ ID NO: 22 - protein, 8 aa, Artificial sequence
  HCDR2
INPYNGGT

SEQ ID NO: 23 - protein, 16 aa, Artificial sequence
  HCDR3
ARDLWNDDVDYYGMDV

SEQ ID NO: 24 - protein, 16 aa, Artificial sequence
  HCDR3
ARDVWQQGGYYYYMDV

SEQ ID NO: 25 - protein, 6 aa, Artificial sequence
  LCDR1
QSISTY

SEQ ID NO: 26 - protein, 6 aa, Artificial sequence
  LCDR1
QSISSY

SEQ ID NO: 27 - protein, 6 aa, Artificial sequence
  LCDR1
QSVSSY

SEQ ID NO: 28 - protein, 3 aa, Artificial sequence
  LCDR2
AAS

SEQ ID NO: 29 - protein, 3 aa, Artificial sequence
  LCDR2
GAS

SEQ ID NO: 30 - protein, 3 aa, Artificial sequence
  LCDR2
DAS

SEQ ID NO: 31 - protein, 3 aa, Artificial sequence
  LCDR2
TAS

SEQ ID NO: 32 - protein, 9 aa, Artificial sequence
  LCDR3
QQSYSTPLT

SEQ ID NO: 33 - protein, 8 aa, Artificial sequence
  HCDR1
  misc_feature (1)..(1): Xaa can be any naturally occurring amino acid
  misc_feature (3)..(3): Xaa can be any naturally occurring amino acid
  misc_feature (5)..(7): Xaa can be any naturally occurring amino acid
XYXFXXXY

SEQ ID NO: 34 - protein, 8 aa, Artificial sequence
  HCDR2
  misc_feature (1)..(1): Xaa can be any naturally occurring amino acid
  misc_feature (3)..(8): Xaa can be any naturally occurring amino acid
XNXXXXXX

SEQ ID NO: 35 - protein, 16 aa, Artificial sequence
  HCDR3
  misc_feature (4)..(4): Xaa can be any naturally occurring amino acid
  misc_feature (6)..(9): Xaa can be any naturally occurring amino acid
  misc_feature (11)..(11): Xaa can be any naturally occurring amino acid
  misc_feature (16)..(16): Xaa can be any naturally occurring amino acid
ARDXWXXXXDXYGMDX

SEQ ID NO: 36 - protein, 6 aa, Artificial sequence
  LCDR1
  misc_feature (1)..(3): Xaa can be any naturally occurring amino acid
  misc_feature (5)..(6): Xaa can be any naturally occurring amino acid
XXXSXX

SEQ ID NO: 37 - protein, 3 aa, Artificial sequence
  LCDR2
  misc_feature (1)..(3): Xaa can be any naturally occurring amino acid
XXX

SEQ ID NO: 38 - protein, 9 aa, Artificial sequence
  LCDR3
  misc_feature (9)..(9): Xaa can be any naturally occurring amino acid
QQSYSTPLX

SEQ ID NO: 39 - protein, 25 aa, Artificial sequence
  HFR1
  misc_feature (1)..(3): Xaa can be any naturally occurring amino acid
  misc_feature (5)..(6): Xaa can be any naturally occurring amino acid
  misc_feature (18)..(18): Xaa can be any naturally occurring amino acid
XXXLXXSGAEVKKPGASXKVSCKAS

SEQ ID NO: 40 - protein, 17 aa, Artificial sequence
  HFR2
  misc_feature (1)..(1): Xaa can be any naturally occurring amino acid
  misc_feature (12)..(12): Xaa can be any naturally occurring amino acid
XHWVRQAPGQGXEWMGW

SEQ ID NO: 41 - protein, 38 aa, Artificial sequence
  HFR3
  misc_feature (12)..(12): Xaa can be any naturally occurring amino acid
  misc_feature (14)..(14): Xaa can be any naturally occurring amino acid
  misc_feature (16)..(16): Xaa can be any naturally occurring amino acid
  misc_feature (18)..(18): Xaa can be any naturally occurring amino acid
  misc_feature (27)..(27): Xaa can be any naturally occurring amino acid
  misc_feature (31)..(31): Xaa can be any naturally occurring amino acid
NYAQKFQGRVTXTXDXSXSTAYMELSXLRSXDTAVYYC

SEQ ID NO: 42 - protein, 11 aa, Artificial sequence
  HFR4
  misc_feature (3)..(3): Xaa can be any naturally occurring amino acid
  misc_feature (6)..(6): Xaa can be any naturally occurring amino acid
WGXGTXVTVSS

SEQ ID NO: 43 - protein, 26 aa, Artificial sequence
  LFR1
  misc_feature (1)..(3): Xaa can be any naturally occurring amino acid
  misc_feature (9)..(10): Xaa can be any naturally occurring amino acid
  misc_feature (13)..(13): Xaa can be any naturally occurring amino acid
  misc_feature (15)..(15): Xaa can be any naturally occurring amino acid
  misc_feature (17)..(17): Xaa can be any naturally occurring amino acid
  misc_feature (19)..(19): Xaa can be any naturally occurring amino acid
  misc_feature (21)..(22): Xaa can be any naturally occurring amino acid
XXXLTQSPXXLSXSXGXRXTXXCRAS

SEQ ID NO: 44 - protein, 17 aa, Artificial sequence
  LFR2
  misc_feature (2)..(2): Xaa can be any naturally occurring amino acid
  misc_feature (10)..(10): Xaa can be any naturally occurring amino acid
  misc_feature (13)..(13): Xaa can be any naturally occurring amino acid
  misc_feature (17)..(17): Xaa can be any naturally occurring amino acid
LXWYQQKPGXAPXLLIX

SEQ ID NO: 45 - protein, 36 aa, Artificial sequence
  LFR3
  misc_feature (1)..(4): Xaa can be any naturally occurring amino acid
  misc_feature (6)..(6): Xaa can be any naturally occurring amino acid
  misc_feature (8)..(8): Xaa can be any naturally occurring amino acid
  misc_feature (18)..(18): Xaa can be any naturally occurring amino acid
  misc_feature (24)..(24): Xaa can be any naturally occurring amino acid
  misc_feature (27)..(29): Xaa can be any naturally occurring amino acid
  misc_feature (31)..(31): Xaa can be any naturally occurring amino acid
XXXXGXPXRFSGSGSGTXFTLTIXSLXXXDXATYYC

SEQ ID NO: 46 - protein, 11 aa, Artificial sequence
  LFR4
  misc_feature (3)..(3): Xaa can be any naturally occurring amino acid
  misc_feature (6)..(8): Xaa can be any naturally occurring amino acid
FGXGTXXXIKR

SEQ ID NO: 47 - protein, 123 aa, Artificial sequence
  VH
  misc_feature (1)..(3): Xaa can be any naturally occurring amino acid
  misc_feature (5)..(6): Xaa can be any naturally occurring amino acid
  misc_feature (18)..(18): Xaa can be any naturally occurring amino acid
  misc_feature (26)..(26): Xaa can be any naturally occurring amino acid
  misc_feature (28)..(28): Xaa can be any naturally occurring amino acid
  misc_feature (30)..(32): Xaa can be any naturally occurring amino acid
  misc_feature (34)..(34): Xaa can be any naturally occurring amino acid
  misc_feature (45)..(45): Xaa can be any naturally occurring amino acid
  misc_feature (51)..(51): Xaa can be any naturally occurring amino acid
  misc_feature (53)..(58): Xaa can be any naturally occurring amino acid
  misc_feature (70)..(70): Xaa can be any naturally occurring amino acid
  misc_feature (72)..(72): Xaa can be any naturally occurring amino acid
  misc_feature (74)..(74): Xaa can be any naturally occurring amino acid
  misc_feature (76)..(76): Xaa can be any naturally occurring amino acid
  misc_feature (85)..(85): Xaa can be any naturally occurring amino acid
  misc_feature (89)..(89): Xaa can be any naturally occurring amino acid
  misc_feature (100)..(100): Xaa can be any naturally occurring amino acid
  misc_feature (102)..(105): Xaa can be any naturally occurring amino acid
  misc_feature (107)..(107): Xaa can be any naturally occurring amino acid
  misc_feature (112)..(112): Xaa can be any naturally occurring amino acid
  misc_feature (115)..(115): Xaa can be any naturally occurring amino acid
  misc_feature (118)..(118): Xaa can be any naturally occurring amino acid
XXXLXXSGAEVKKPGASXKVSCKASXYXFXXXYXHWVRQAPGQGXEWMGWXNXXXXXXNYAQKFQGRVTXTXDXSXSTAYMELSXLRSXDTAVYYCARDXWXXXXDXYGMDXWGXGTXVTVSS

SEQ ID NO: 48 - protein, 108 aa, Artificial sequence
  VL
  misc_feature (1)..(3): Xaa can be any naturally occurring amino acid
  misc_feature (9)..(10): Xaa can be any naturally occurring amino acid
  misc_feature (13)..(13): Xaa can be any naturally occurring amino acid
  misc_feature (15)..(15): Xaa can be any naturally occurring amino acid
  misc_feature (17)..(17): Xaa can be any naturally occurring amino acid
  misc_feature (19)..(19): Xaa can be any naturally occurring amino acid
  misc_feature (21)..(22): Xaa can be any naturally occurring amino acid
  misc_feature (27)..(29): Xaa can be any naturally occurring amino acid
  misc_feature (31)..(32): Xaa can be any naturally occurring amino acid
  misc_feature (34)..(34): Xaa can be any naturally occurring amino acid
  misc_feature (42)..(42): Xaa can be any naturally occurring amino acid
  misc_feature (45)..(45): Xaa can be any naturally occurring amino acid
  misc_feature (49)..(56): Xaa can be any naturally occurring amino acid
  misc_feature (58)..(58): Xaa can be any naturally occurring amino acid
  misc_feature (60)..(60): Xaa can be any naturally occurring amino acid
  misc_feature (70)..(70): Xaa can be any naturally occurring amino acid
  misc_feature (76)..(76): Xaa can be any naturally occurring amino acid
  misc_feature (79)..(81): Xaa can be any naturally occurring amino acid
  misc_feature (83)..(83): Xaa can be any naturally occurring amino acid
  misc_feature (97)..(97): Xaa can be any naturally occurring amino acid
  misc_feature (100)..(100): Xaa can be any naturally occurring amino acid
  misc_feature (103)..(105): Xaa can be any naturally occurring amino acid
XXXLTQSPXXLSXSXGXRXTXXCRASXXXSXXLXWYQQKPGXAPXLLIXXXXXXXXGXPXRFSGSGSGTXFTLTIXSLXXXDXATYYCQQSYSTPLXFGXGTXXXIKR